European Patent Specification EP 3 572 509 B1, published September 20, 2023. Title: A primer set, a probe, a kit and a method for detecting Mycobacterium kansasii. Applicant: Kaneka Corporation Kyokuto Pharmaceutical Industrial Co., Ltd. The sequence listing filed with the application follows.

SEQUENCE LISTING (44 sequences)

SEQ ID NO: 1 - DNA, 333 bp, Mycobacterium kansasii type I
gccatcccgcaagtccggtcgctgacgagtgagaacgaggaggagccatgggggatacctaccgcgaccccgtcgaccacctgcatacgacgcgtccgctggccggtgagtcactgatcgacgtgctgcactggcccgggtatctgctggtggtggccggggttatcggcggtgtcggatctcttgccgccttcggtaccgggcatgactcccagggcatggtcgccggtgtcgcagcgctcgtggtcacggtggccgggctggtgtggctggccgtcgagcaccggcgggtgcgccgaatcgccgaacggtggtatgccgaacatcccgagg

SEQ ID NO: 2 - DNA, 475 bp, Mycobacterium kansasii type I
tcgccgtcgggggcgccgttcaccgggttcaccggctccatgaccggcagcgcgccgtcgggatcgcaaatctcgagtaaccgcgacacagcccggctcggcaccagcgcccaccggatgtctgccgccgagcagaccacgttgattcggtgaagagcggaaaacccggcagtaccaatgaattccaggtggcgtaggtccagggtcagccaccggcaagaccgcacgcactgctgcacgtatccggtgagctgatcggcattggcggcgtcgagctcaccttccacggtgatcacgccggccgacggcccatagctggcagtgaagtcagcggttccgcatttctgccaggattggatcacagacaatcgtggactccatccatcgagcgtttgttgctgtcgaccacgccgcgtctgcgcgggaccgctatacagggagtttgccttcctggcgaccctgacgcactgacagg

SEQ ID NO: 3 - DNA, 20 bp, Artificial
  Primer
tgaattccaggtggcgtagg

SEQ ID NO: 4 - DNA, 20 bp, Artificial
  Primer
atcctggcagaaatgcggaa

SEQ ID NO: 5 - DNA, 20 bp, Artificial
  Primer
cgcaaatctcgagtaaccgc

SEQ ID NO: 6 - DNA, 20 bp, Artificial
  Primer
cgctcttcaccgaatcaacg

SEQ ID NO: 7 - DNA, 20 bp, Artificial
  Primer
tcgtggactccatccatcga

SEQ ID NO: 8 - DNA, 20 bp, Artificial
  Primer
ggagctacgtcctgtcagtg

SEQ ID NO: 9 - DNA, 338 bp, Mycobacterium kansasii type II
gccatcgtgtcccgcgagtccggccgctgacgagtgagaacgaggaggaaccatgggggacacctaccacgaccccgtcgaccacctgcatacgacgcggccgctggccggcgagtcactgatcgacgtgctgcactggcccgggtacctgctggtggtggccggggttatcggcggtgtcgggtctcttgccgccttcggcaccgggcatcactcccagggcatggtcgccggtgtcgcggcgctcgtggtcacggtggccgggctggtgtggctggccgtggagcaccggcgggtgcgccgaatcgccgagcggtggtatgccgaacacccggagg

SEQ ID NO: 10 - DNA, 476 bp, Mycobacterium kansasii type II
tcgccgtcgggggcgccgttcacccggttcaccggctccatgaccggcagcgcgccgtcgggatcgcaaatttccagtaaccgcgatacggcccggctcggcaccatcgcccactgggtgtcggccgccgagcagaccacgttgattcggtgaagagcggaaaacccggcagtcccaataaattccagacgccgtaggtccagggtcagccaccggcagtacttcacgcattgctggacgtatccggcgagatggtcggcgttggcggcgtcgagctcaccttctacggtgaccacgccggacgacgaaccatagctggcggtgaagtcagcggttccgcatttctgccaggattggatcacagacaatcgtggactccatccatcgaacattctttggtgtcgaccacgtcgagtgtgcgctgcgccgcttaagcagggaatttgcctccctcgcgaccctgacgcactgacagg

SEQ ID NO: 11 - DNA, 338 bp, Mycobacterium kansasii type III
gccatccggtcccgcgagtccgatcgctgacgagtgagaacgaggaggagccatgggggacacctaccgcgaccccgtcgaccacctgcatacgacgcggccgctggccggcgagtcgctgatcgacgtgctgcactggcccgggtacctgctggtggtggccggggttatcggcggtgtcggatctcttgccgccttcggcaccgggcatgactcccagggcatggtcgccggcgtcgcggcgctcgtggtcacggtggccgggctggtgtggctggccgtcgagcatcggcgggtgcgtcgaatcgccgagcggtggtatgccgaacatcccgagg

SEQ ID NO: 12 - DNA, 466 bp, Mycobacterium kansasii type III
ccgccgtcgggggtgtcgttcaccggctccatgaccggcagcgcgccgtcgggatcgcaaatctccagtaaccgcgacacggcccggctcggcaccatcgcccactgggtgtccgccgccgaacagaccacgttgattcggtgaagagcggaaaacccggcagtcccaataaattccagacgccgtaggtccagggtcagccaccggcaataccttgcgcactgctggacgtatccggcgagctgatcggcgttggcggcgtcgagctcaccctctacggtgaccacgccggccgacggacgatagctggcagtgaagtcagcggttccgcatttctgccaggattggatcacagacaatcgtggactccatccatcgagcatgtgttgctgtcgaccacgtcgcgtctgcagcgggccgttatgcagggagtttgcctccctggcgaccctgacgcagtgacagg

SEQ ID NO: 13 - DNA, 340 bp, Mycobacterium kansasii type IV
tccacatcctgtcccgtgagtcccgtcgctgacgagagagaacgaggaggagccatgggggacacctaccgcgaccccgtcgaccacctgcatacgacgcggccgctggccggcgagtcactgatcgacgtgctgcactggcctgggtacctgttggtggtggcgggggtgatcggtggtgtcggatctcttgctgccttcggcaccggccatcacgtcgaaggcatggtcgccggcgtcgcggcgctcgtcgtcacggtggccgggctggtgtggctggccgtcgagcaccggcgggtacgcaggatcgccgagcggtggtacgccgaacaccccgagg

SEQ ID NO: 14 - DNA, 477 bp, Mycobacterium kansasii type IV
tcgccgtcgggggcgccgtttaccgggttcaccggctccatgaccggcagcgcgccgtcgggatcgcaaatctccagtaaccgcgacacggcccggctcggcaccatcgcccactgggtgtccgccgccgagcagaccacgttgattcggtgaagggcggaaaacccggcagtgccaatgaattccagacgccgtaggtccaggatcagccaccggcaagacctcacgcactgctggacgtatccggccagctgatcggcattggcggcgtcgagctcaccttctacggtgatcacgccggccgacggcccatagctggcagtgaagtcagcggttccgcatttctgccaggattggatcacagacaatcgtggactccatccatcgaacattcgttggtgtcgaccacgtcgagtgtgcgctgcgtcgctttacgcagggagtttgcctccctcgcgaccctgacgcactgacagg

SEQ ID NO: 15 - DNA, 339 bp, Mycobacterium kansasii type V
gccatcctgtcccgcgagtccggccgctgacgagtgagaacgaggaggagccatgggggacacctaccgcgaccccgtcgaccacctgcatacgacgcggccgctggccggcgagtcactgatcgacgtgctgcactggccccgggtatctgctggtggtggccggggttatcggcggtgtcggatctcttgccgccttcggcaccgggcataactcccagggcatggtcgccggtgtcgcggcgctcgtggtcacggtggccgggctggtgtggctggccgccgagcaccggcgggtgcgccgaatcgccgagcggtggtatgcggaacaccccgagg

SEQ ID NO: 16 - DNA, 476 bp, Mycobacterium kansasii type V
tcgccgtcgggggcaccgttcaccgggttcaccggctccatgaccggcagcgcgccgtcgggatcgcaaatctccagtaaccgcgacacggcccggctcggcaccatcgcccactgggtgtccgccgccgagcagaccacgttgattcggtgaagagcggaaaacccggcagtcccaataaattccaggcgccgtaggtccagggtcagccaccggcaatacctcacgcactgctggacgtatccggcgagctgatcggcgttggcggcgtcgagctcaccttctacggtgaccacgccggccgacggaccatagctggcagtgaagtcagcggttccgcatttctgccaggattggatcacagacaatcgtggactccatccatcgaacattcgttggtgtcgaccacgtcgagtgtgcgctgtgcggcttacgcagggagtttgcctccctcgcgaccctgacgcactgacagg

SEQ ID NO: 17 - DNA, 5001 bp, Mycobacterium kansasii type I
ggcgatggctcgcttcgtcgagaccttcgtcagggtgttgggcgacccggagctgccgcatctgttcttcgtcgagggcggcgctttggcggtggagaacgccctcaaggtcgcattcgactggaagagccgccacaaccaggcgcgcggcatcgatccggcgctcggcacccgggtgctgcacttgagcggggcatttcacggccgcagcggctataccctgtcgctgaccaacaccaaacccgttacggtggcccgctttccgaaattcgactggccgcgcatcgaggcaccctatatccgaccccgagccgacatggatgcgctggaaaccgaggcgctgcggcaggcccgcgcggcattcgaggcgcacccccatgacatcgcctgtttcatcgccgagccgatccagggagaaggcggcgaccgtcacttccggcccgagttcttcgtggcgatgcgccagttgtgtgacgaacacgatgcgctgctgattttcgacgaggtgcagaccggctgtgggctcacgggaaccccttgggcctaccagcaattgggtgtggcgcccgatgtcgtcgccttcggcaagaagacgcaggtgtgcgggatgatggcgggccgccgagtcgacgagatcaccgacaacgtgttcgcggtcaagtcgcggctcaactcgacgtggggcggaaacctggtcgacatggtgcgggcccgccgcatcctggaggtgatcgaaggcgaagggctattcgaacatgcggcccgccagggccgccacctgcgcgcccggctcgacgagcttgcccaggagttcccgggcctggttctgcatccgcgcggccgggggctgatgtgtgccttcagcctgccgaccaccgcggaccgtgacgacgtgatccgccggttgtggcaacgcggggtgatcgtgctgccggcgggtgacgacggggtgcgcttccgtccggcgttgaccgtcacgcgcgccgagatcgacgccgcgatcgccggtgtacgtgccgcattgacggctgtgacctagtcggaccgggtgcaccgtttacctgggctgaccgcggggtatggaaacgttgtactccgcgaacgcgggattggggttcaggaatgcagaagacacgcgagcggtcacccggtgaccgattaggacaggacgacgccgaggttcgcgccgccatccggttcgcagtcctggccgcggccgccggtgtgggttttgtcatcatggcggccttgtgggtcagcacgtgcggtggcgcgggattggacacggtggcctgtggcccgccggagcggaccctgctggccttcggcggcccgctgattctgttggccggtgggatctgggccttcatccgcacctatcaggtgtggcgagcacgcggtacctggtggggatggcacggtgccggatggttcttgttgacgctgatggtggtggccgtgtccatgggcgtgcctcccatcgccggcccggcactggcggttagttggctctgatcccgccatcccgcaagtccggtcgctgacgagtgagaacgaggaggagccatgggggatacctaccgcgaccccgtcgaccacctgcatacgacgcgtccgctggccggtgagtcactgatcgacgtgctgcactggcccgggtatctgctggtggtggccggggttatcggcggtgtcggatctcttgccgccttcggtaccgggcatgactcccagggcatggtcgccggtgtcgcagcgctcgtggtcacggtggccgggctggtgtggctggccgtcgagcaccggcgggtgcgccgaatcgccgaacggtggtatgccgaacatcccgaggtaccgcgccaacggctggccagctagcagctccggctggcgcctcaccgcaaaacccggcggcggttttgttttaccggtggcgccgacggggtatcaggtgtgaaccatgacgagtactggctttgccgcgtcggcactgtcaccccatcatcggggacaggatcacgaaggcaccgacatagattgctgcagcgaccgcgatcaaaaccaccaaggtgatcccggcaatcaccgcgatgcgccggagccggcgcgtccggattgtgtcggtcgcgtccgcctcgtccatggctggttgaatacccggtggcgaccatgaccaaccggttagaacgcgcggcccaaaacgggcctccggaaggcgatcggaaagggaccgaaatcgacagccaaatcgggacccaaatcagtagtagtagtgtcggtcaaaaattgccgggaggccacatgagcgatgccgacgcgcgtcccaacaggcaccaacgcggcgagcgcgccgtcgagctgaaagttgctgcgcgcttggagaatctggcgatcctgcgcaccctggtcggcgccatcggcaccttcgaggacttggatttcgacgcggtcgccgacctgagactggcggtcgacgaagtgtgtacccggctgatccgttccgccacaccgaacgcgaccttgacgctggtggtcgacccgcacgacgacgaactcgtggtggaggcgtccgcgatgtgcgacacccacgacgtcgtggcaccgggcagcttcagctggcatgtcctgacgtcgctggccgacgacgtccagactttccacgacggtcgcatgcccgacgccgccggcagtgtgttcggcattgtgttgacggcccgacgggcggcctctggcaggtgacgccgcgtgctgccggcggttctgcttcacggccgaacgaatacgccgatgtcccggagatgtttcgtgagttggccggttttgaccccgactcaccggatttccagcgccaccgcgacaagatcgtggagcgctgcctaccgctggccgatcacatcgcccggcggttcgagggacgcggcgaaccccgcgacgacctgattcaggtcgcccgggtcggattggtcaacgcggtagtccgcttcgacgtcgagaccgggtcggatttcgtctcgttcgccgtgcccaccatcatgggggaagtccggcggcacttccgggacaacagttggtcagtcaaggttcctcgccggctgaaggaactgcacctgcggttgggcaccgccaccgccgagttgtcgcagcggctcggcagggcgcccaccgctaccgaactcgccgccgaactcggtatggaccgcggcgaggtcgtcgaagggctggtggcgggcagctcttacaacacgctgtcgatcgacagcggtggtggtaacgaagacgacgacgcgcgtgccatcgcggacaccctcggcgacatggatgccggcctggaccggatagaagatcgcgagtcgcttcgcccgctgctcgaggcgctgcccgagcgcgagcgaacggtgttgatcctgaggtttttcgagtcgatgacgcagacccagatcgccgagcgggtcggcatctcccagatgcacgtgtcccggctgctggccaagtcgctagcgcggctccgcgaccagctcgagtaggcgcaggtcgccgtcgggggcgccgttcaccgggttcaccggctccatgaccggcagcgcgccgtcgggatcgcaaatctcgagtaaccgcgacacagcccggctcggcaccagcgcccaccggatgtctgccgccgagcagaccacgttgattcggtgaagagcggaaaacccggcagtaccaatgaattccaggtggcgtaggtccagggtcagccaccggcaagaccgcacgcactgctgcacgtatccggtgagctgatcggcattggcggcgtcgagctcaccttccacggtgatcacgccggccgacggcccatagctggcagtgaagtcagcggttccgcatttctgccaggattggatcacagacaatcgtggactccatccatcgagcgtttgttgctgtcgaccacgccgcgtctgcgcgggaccgctatacagggagtttgccttcctggcgaccctgacgcactgacaggacgtagctccgggcggctgtgaactcaacctgtttcgaggctacccggcgggtgccggggcgacaacgttctccgatctgactcagagaatcgctggtcagacggggtttggctcggtgatcggctacttgatctcggcgagcaccgtgccctgcgtgatggctgccccggcctcgaccgccaggccggtgatgacgccgtccttgtgggcggtgaccgggttttccatcttcatcgcctcaaggaccaccacaagatcgccggtgacgacttcttgtccttcttcgacagcgaccttcaccacggtgccctgcatgggtgcggtcaccgcgtcgccggaggctgccgcgccgctgtgggcgccgcgcttgcgcggcttgggcttgcgccggatgacgccgaccgggtcgcagccgccgccgccggacagcgccaggtcggcgggcagtgacacctcgacccgtcgaccgtcgacctcgacgaccaccttctgccgcggccgggcgtcttcctcgtcgctgggctcgccggcggtgaagggttcgacggtgttgttccactcggtctcgatccaacgggtgtgcaccgagaagccgtcctggtcgccgatgaacgccgggtcggccaccaccgcccggtggaaggggatgacggtggccagaccctccacctcgaattcgtccagcgcgcgacgcgcgcgggccagcgcctcggcgcggtcggcgccgtggacgatcagcttggccagcatcgagtcgaactggccgccgatcaccgagccggtctccacgccggaatccagccggacgcccgggccgctgggcgggtggaatttggtcaccggtccgggcgcgggcaagaatccgcgcccggcgtcctcgccgttgatccggaactcgatggcgtgcccgcggggggtggggtcctcggtgatgtccagcttttcgccgttggcgatcttgaactgctgcagcaccaagtcgataccggcggtt

SEQ ID NO: 18 - DNA, 5034 bp, Mycobacterium kansasii type II
ggcgatggcgcgcttcgtcgagaccttcgtcagggtgttgggcgacccggcgctgccgcatctgttcttcgtcgagggcggcgctttggcggtggagaacgccctcaaggtcgcattcgactggaaaagccgccacaaccaggcccgcggcatcgatccggcgctgggcacccgggtgctgcacttgagcggcgcatttcacggccgcagcggctacaccctgtcgctcaccaacaccaaacccgtcaccgtggcccgcttcccgaaattcgactggccgcgcatcgacgcgccccatatccggccggggttaaccgagtcggccatggctgcgctggaggccgaggcgctgcggcaggcccgcgcggcattcgaggcgcacccccacgacatcgcctgtttcatcgccgagccgatccagggagaaggcggcgaccgccacttccgggccgagttcttcgcggcgatgcggcagttgtgtgacgaacacgacgcgctgctgatatttgacgaggtgcagaccggctgtggaatcaccggaaccccttgggcttaccagcaattggccgtggcgcccgatgtcgtggccttcggcaagaagacgcaggtctgtggggtgatggcaggccgccgcgtcgacgaggtcaccgacaacgtgttcgcggtcaagtcgcggctcaactcgacgtggggcggaagcctggtcgacatggtgcgggcccgccgcatcctggaggtgatcgaaaacgacggactcttcgaacatgcggcccggcagggccgacacctgcgcgcccggctcgacgagcttgcccaggagttcccgggcctggtactggatccgcgcgggcgggggctgatgtgtgccttcagcctgccgaccaccgcggaccgtgacgacgtgatccgccagttgtggcaacgcgcggtgatcgtgctgccggccggtgacgacggggtgcgtttccgtccggccttgaccgtcacgcgcgccgagatcgatgccgcgatcgccggtgtacgtgccgcattgacggctgtgacgtagtcggacctggtcggacctggtcgcaccgtttgcctgggctgagcgcggggtatggaaacgttgtactccgcgaacgcgggattggggttttcaggatgcagaagacacgcgaacggtcacccggtgaccgactaggacaagacgacgccgaggttcgcgccgccatccggttcgcagtcctggccgccggcgctggtgcggggtttgtcatcatggcggccttgtgggtcagcacgtgcggcggcgcggccgtggacacggtggcctgtggcccgccggagcggaccctgctggccttcggcggcccgctgattctgttggccggtggcatctgggccttcatccgcacctatcaggtgtggcgagcccgcggtacctggtggggatggcacggtgccggatggttcttgttgacgctgatggtggtggccgtgtccatgggcgtgcctcccatcgccggcccggcactggcggttagttggctctgaccccgccatcgtgtcccgcgagtccggccgctgacgagtgagaacgaggaggaaccatgggggacacctaccacgaccccgtcgaccacctgcatacgacgcggccgctggccggcgagtcactgatcgacgtgctgcactggcccgggtacctgctggtggtggccggggttatcggcggtgtcgggtctcttgccgccttcggcaccgggcatcactcccagggcatggtcgccggtgtcgcggcgctcgtggtcacggtggccgggctggtgtggctggccgtggagcaccggcgggtgcgccgaatcgccgagcggtggtatgccgaacacccggaggtaccgcgccaacggctggccagctagcggcttccagtgccggttgacgccgcgccacaaaaccgggcgacggttttgttttaccggtggcgtcgacggggtatcaggtgtgaaccatgacgagtactggctttgccgcgtcggcgctgtcaccccatcatcggggacagaatcacgaaggcaccgacatagattgctgctgcgaccgcgatgaaaaccaccaaggtgatcacggcgatcacggcgacgcgccggagccggcgcgtccggattgtgtcggtcccgtccgcctcgtccatggctggttgaatacccggtggcggccatgaccaaccggttagaacgcgcggcccaaaacgggcctccgggaggcgatcggaaagggaccgaaatcgacagtcaactcgggacccaaatcagtagtagtagtgtcggtcaaaaattgccgggaggccacatgagcgatgccgatgcgcgtcccaacaggcaccaacgcggcgagcgcgccgtcgagctgaaggttgctgcgcgcttggagaatttggcgatcctgcgcaccctggtcggcgccatcggcaccttcgaggacttggatttcgacgcggtcgccgacctgagactggcggtcgacgaagtgtgtacccggctgatccgttccgccacaccgaacgcgaccttgacgctggtggtcgacccgcgcgacgacgaactcgtggtggaggcgtccgcgatgtgcgacacccacgacgtagtggcgccgggcagcttcagctggcatgtcctgacgtcgctggccgacgacgtccagactttccacgacggccgcatgcctgacgccgccggcagtgtgttcggcattgtgttgacggcccgacgggcggcctctggcaggtgacgccgcgtgctgccggcggttctgcttcacggccgaacgaatacgccgatgtcccggagatgtttcgtgagttggccggttttgaccccgactcaccggatttccagcgccaccgcgacaagatcgtggagcgctgcctgccgctggccgatcacatcgcccggcggttcgagggacgcggcgaaccccgcgacgacctgattcaggtcgcccgggtcggactggtcaacgcggtagtccgcttcgatgtcgataccgggtcggacttcgtctcgttcgccgtgcccaccatcatgggggaagtcaggcggcacttccgggacaacagctggtcagtcaaggttcctcgccggctgaaggaactgcacctgcggttgggcaccgccaccgccgagttgtcgcagcggctcggcagggcgcccaccgccaccgaactcgccgccgaactcgggatggaccgcggcgaggtggtcgaggggctggtggcgggcagctcttacaacacgctgtccatcgacagcggtggtggtaacgaagacgacgacgcccgcgccatcgcggacaccctcggcgacatggatgccggcctggaccgaatcgaagatcgcgagtcgctgcgcccgctgctcgaggcgctgcccgagcgcgagcgaacggtgttgatcctcaggtttttcgaatcgatgacgcagacccagatcgccgagcgggtcggcatctcccagatgcacgtgtcccggctgctggccaagtcgctagcgcggctccgcgaccagctcgagtaggcgcaggtcgccgtcgggggcgccgttcacccggttcaccggctccatgaccggcagcgcgccgtcgggatcgcaaatttccagtaaccgcgatacggcccggctcggcaccatcgcccactgggtgtcggccgccgagcagaccacgttgattcggtgaagagcggaaaacccggcagtcccaataaattccagacgccgtaggtccagggtcagccaccggcagtacttcacgcattgctggacgtatccggcgagatggtcggcgttggcggcgtcgagctcaccttctacggtgaccacgccggacgacgaaccatagctggcggtgaagtcagcggttccgcatttctgccaggattggatcacagacaatcgtggactccatccatcgaacattctttggtgtcgaccacgtcgagtgtgcgctgcgccgcttaagcagggaatttgcctccctcgcgaccctgacgcactgacaggacgtagctccgggcggctgtgaactcaacctgttttgaggctacccggcgggtgccggggcgacaacgttctccgatccgactcagagaatcgctggtcaggcggggttggcgcggtgagcggctacctgatctcggcgagcaccgtgccctgggtgattgcggccccggcttcgacggccaatccggtgatgacgccgtccttgtgcgcggtgaccgggttctccatcttcatcgcctccaggacaaccaccagatcgcccgtcaccacttcctgaccttcttcgaccgcgaccttcaccacggtcccctgcatgggcgcggtcacagcgtcgccggaggcagccgcaccgctgtgggcgccacgcttgcgcggcttgggcttgcgccggataacaccgaccgggtcgcacccgccaccgccggacagtgcgagatcggcaggcagtgacacctcgacccggcggccgtcgacctcgacgaccaccttctgccgcggccgggcgtcctcttcgtcgctcggctcgccgccggtgaagggttcgacggtgttgttccactcggtctcgatccagcgggtgtgcaccgagaatccgtgctcgtcgccgatgaacgccgggttggacaccaccgcccggtggaaggggatgaccgtcgccagaccctcgacttcgaattcggccagcgcccggcgggcacgcgccagcgcctcggcgcggtcggcgccgtggacgatcagcttggccagcatcgagtcgaactggccgccgatcaccgagccggtttccacgccggagtccagccgcacgcccgggccgctgggcgggtggaacttggtcaccgggccgggtgcgggcaaaaagccgcgcccggcgtcctcgccgttaatccggaactcgatggcgtgcccgcgcggggtggggtcctcggtgatgtcgagcttgtcgccgttggcgatcttgaactgctgtagcaccaagtcgatgccggcggtt

SEQ ID NO: 19 - DNA, 5031 bp, Mycobacterium kansasii type III
ggtgatggctcgattcgtcgagaccttcgtcagggtgttgggcgacccggcgctgccgcatcttttcttcgtcgagggcggcgcgttggcggtggagaacgccctcaaggtcgcattcgactggaaaagccgctacaaccaggcgcatggcatcgatccggcgctcggcacccgggtactgcacttgagcggggcatttcacggccgcagcggctacaccctgtcgctcaccaacaccaaagccgtcacggtggcccgttttccgagattcgattggccgcgcatcgacgcgccgtatatccgacccggtttaagcgagtcggccatcgatgcgctggagggcgaggcgctgcggcaggcccgcgcggcattcgaggcgcatccacatgacatcgcctgtttcatcgccgagcccgtccagggcgaaggcggggaccgccacttccggcccgagttcttcaccgcgatgcgccggctctgcgacgaacacgatgcgctgctgattttcgacgaggtgcagaccggctgcgggatcaccggaaccccgtgggcgtaccagcaactgggtgtagcgcccgatgtcgtggcattcggaaaaaagacccaggtgtgcggggtgatggcgggccgccgagtcgacgaggtcaccgacaacgtgttcgccgtcacgtcgcggctcaactcgacgtggggcggaaacctggtcgacatggtgcgggcccgccgcatcctggaggtgatcgaaagcgacgggctcttcgaacatgcggcccggcagggccgccacctgcgtgcccggctcgacgagcttgcccaggagttccggggcctggttctccatccgcgcggccgggggttgatgtgtgccttcagcctgccgaccaccgcggaccgtgacgacgtgatccgccggctctggcaacgcgcggtgattgtgctaccgacgggtgacgacggggtgcgcttccgcccggcgttgaccgtcacgcgcgccgagatcgatgccgcgatcgctggtgtgcgtgcagccttgacggctgtgacctaggtgtggcccaggtgtggaccaagccgcaccgtttgcctgggctgaccgcggggtatggaaacgttgtactccgcgaatgcgggatggggttcaggaatgcagaacacacgcgaacggtcaccgggtgaccgactaggacaggacgacgccgaagttcgcgccgccatccggttcgcagtcctggccgcgggcgctggtgtggggtttgtcatcatggcggccttgtgggtcagcacctgcggcggcagagcgggcctggacacggtggcctgtggcccgccggaacggaccctgctggccctcggcggcccgctgattctgttggccggcggaatctgggccttcatccgcacctatcaggtgtggcgagcccgcggtacctggtggggatggcatggcgccggatggttcttgttgacgctgatggtggtggccgtgtccatgggcgtggctcccatcgccggcccggcactggcggttggttggctctgatcccgccatccggtcccgcgagtccgatcgctgacgagtgagaacgaggaggagccatgggggacacctaccgcgaccccgtcgaccacctgcatacgacgcggccgctggccggcgagtcgctgatcgacgtgctgcactggcccgggtacctgctggtggtggccggggttatcggcggtgtcggatctcttgccgccttcggcaccgggcatgactcccagggcatggtcgccggcgtcgcggcgctcgtggtcacggtggccgggctggtgtggctggccgtcgagcatcggcgggtgcgtcgaatcgccgagcggtggtatgccgaacatcccgaggtcccgcgccaacggctggccagctagcagcttccagtgccggctggcgcctcatcgcaagaaccgagcgacggttttgttttaccagtggcaccgacggggtatcaggtgtgaaccatgacgagtactggcattgccgcgtcggcgctgtcaccccatcatcggggacagaatcacgaaggcaccgacatagattgctgcagcgaccgcgatcaaaaccaccaaggtgaccccggcgaccaccgcgatgcggcggagccggcgcgtccggattgtgtcggtcacgtccgcctggtccatggctggttgaatacccggtggcgaccatgaccaaccggttggaacgcgcggcccaaaacgggcctccgggaggcgatcggaaagggaccgaaatcgacagccaaatcgggacccacatcagtagtagtagtgtcggtcaaaaattgccgggaggccacatgagcgatgccgacgcgcgtcccaacaggcaccaacgcggcgaccgcgccgtcgagctgaacgttgctgcgcgcttggagaatctggcgatcctgcgcaccctggtcggcgccatcggcaccttcgaggacttggatttcgatgcggtcgccgacctgagactggcggtcgacgaagtgtgtacccggctgatccgttccgccacaccgaacgcgaccttgacgctggtggtcgacccgcgcgacgacgaactcgtggtggaggcgtccgcgatgtgcgacacccacgacgtggtggcacccggcagcttcagctggcatgtgctgacatcgctggccgacgacgtccagacgttccacgacggtcgtatgcccgacgccgccggcagtgtgttcggcattgtgttgacggcccgacgggcggcctctggcaggtgacgccgcgtactgccggcggttctgcttcacggccgaacgaatacgccgatgtcccggagatgtttcgtgagttggccggttttgaccccgactcgccggatttccagcgccaccgcgacaaaatcgtggagcgctgcctgccgctggccgatcacatcgcccggcggttcgagggacgcggcgaaccccgcgacgacctgattcaggtcgcccgggtcggactggtcaacgcggtagtccgcttcgatgtcgagaccgggtcggatttcgtctcgttcgccgtgcccaccatcatgggggaagtccggcggcacttccgggacaacagttggtcggtcaaggttcctcgccggctgaaggaactgcacctgcggttgggcaccgccaccgccgagttgtcccagcggctcggcagggcacccactgccaccgaacttgccgccgaactcggtatggaccgcggcgaggtcgtcgaagggctggtggcgggcagctcttacaacacgctgtcaatcgacagcggtggcggtaacgaagacgacgacgcccgagtcatcgcggacaccctcggcgacatggacgccggcctggaccggatcgaagatcgcgagtcgcttcgcccgctgctcgaggcgctgcccgagcgcgagcgaacggtattgatcctcaggtttttcgagtcgatgacgcagacccagatcgccgagcgggtcggaatctcccagatgcacgtgtcccggctgctggccaagtcgctagcgcggctccgcgaccaactcgagtaggcgcacgccgccgtcgggggtgtcgttcaccggctccatgaccggcagcgcgccgtcgggatcgcaaatctccagtaaccgcgacacggcccggctcggcaccatcgcccactgggtgtccgccgccgaacagaccacgttgattcggtgaagagcggaaaacccggcagtcccaataaattccagacgccgtaggtccagggtcagccaccggcaataccttgcgcactgctggacgtatccggcgagctgatcggcgttggcggcgtcgagctcaccctctacggtgaccacgccggccgacggacgatagctggcagtgaagtcagcggttccgcatttctgccaggattggatcacagacaatcgtggactccatccatcgagcatgtgttgctgtcgaccacgtcgcgtctgcagcgggccgttatgcagggagtttgcctccctggcgaccctgacgcagtgacaggacgtggctccgggcggctgtgaactcaacctgtttcgaggctacccggcgggtgccggggcgacaacgttctccgatccgactcagagaatcgctggtcagacgggggcggccggcagtgagcggctacttgatctcggcgagcaccgtgccttgggtgatggcggccccggcctcgaccgccaggccggtgatgacgccgtccttatgcgcggtgaccgggttctccatcttcatcgcctccagcaccaccacgagatcgccggtcaccacctcctggccttcttcgaccgcgaccttcaccacggtgccctgcatgggcgcggtaacggcgtcgcccgatgctgccgcaccgctgtgggcaccacgcttgcgcggcttgggcttgcgtcggataacgccaaccgggtcgcacccgccgccgccggacagtgcgaggtcggccggcagcgacacctcgacccggcggccgtcgacctcgacgaccaccttctgccgcggccgggcgtcttcctcgtcgctgggctcgccggcggtgaagggttcgacggtgttgttccactcggtctcgatccagcgggtgtgcaccgagaagccgtgctcgtcgccgatgaacgccgggtcggacaccaccgcccggtggaaggggatgacggtggccagaccctccacctcgaattcgtccagcgcgcggcgcgcgcgggccagcgcctcgccgcggtcggcgccgtgaacgatcagcttggccagcatcgagtcgaactggccgccgatcaccgagccggtctccacgccggagtccagccgcacgcccgggcccgcgggcgggtggaacttggtcaccgggccgggggcgggcaggaagccccggccggcgtcctcgccgttgatccggaactcgatggcgtgcccgcgcggggtgggatcctcggtgatgtcgagcttgtcgccgttggcgatcttgaactgctgcagcaccaggtcgatgccggcggtt

SEQ ID NO: 20 - DNA, 5039 bp, Mycobacterium kansasii type IV
gccatggctcgcttcgtcgagaccttcgtcagggtgttgggcgacccggcgctgccgcatctgttcttcgtcgaaggcggcgctgtggcggtggagaacgccctcaaggtcgcattcgactggaagagccgccacaaccaggcgcgcggcgtcgatccggcgctcggcacccgggtactgcacctgagcggggcattccacggccgcagcggctacaccctgtcgctcaccaacaccaaacccgtcaccgtggcccgcttcccgaaattcgattggccgcgcatcgacgcaccctatgtccgaccgggttcaagcgagtcggccatggctgcgctggaggccgagtcgctgcggcaggcccgcgcggcattcgaggcgcatccccatgacatcgcctgcttcatcgccgagcccatccagggagaaggcggcgcccgccacttccgggccgagttcttcgcggcgatgcgccagttgtgtgacgaacacgatgcgctgctgattttcgacgaggtgcagaccggctgtgggataaccggaaccccttgggcttaccagcaattgggcgtggcgcccgatgtcgtggccttcggcaagaagacgcaggtgtgcggggtgatggcaggccgccgcgtcgacgaggtcaccgacaacgtgttcgcggtcaagtcgcggctcaactcgacgtggggcggaaacctggtcgatatggtgcgggcccgccgcatcctggaggtgatcgaaaacgacgggctcttcgaacatgcggcccggcagggccgccacctgcgcgcccggctcgacgagcttgctcaggagttcccgggcctggttctggatccgcgcggccgggggctgatgtgtgccttcagcctgccgaccaccgcggaccgtgacgacgtgatccgccggttgtggcaacgcgcggtgatcgtgctgccggccggtgacgacggggtgcgtttccgtccggcgttgaccgtcacgtgctccgagatcgatgccgcgatcgccggtgtacgtgaggcgttgccggctgtgacctagtcggacctagtcggacctggtcggacctggtcgcactgtttgcctgggctgaccgcggggtatgaagatcttgtactccgcgaacgcgggattggggtttcaggatgcagaagacgcgcgaacggtcacccggtgaccgattaggacaggacgacgccgaggttcgcgccgccatccggttcgctgtcctggccgcgggcgccggtatcgggtttgtcatcatggcggccttgtgggtcagcacgtgcggcggcaaagcgggcctggacacggtggcctgcggcgcgccggagcggaccctgctggccttcggcggcccgctgattctgttggccggcggaatctgggccttcatccgcacctatcaggtgtggcgtgcccgcggtacctggtggggatggcacggcgccggatggtttttgttgacgctgatggtggtggccgtgtccatgggggtgcctcccatcgtcggcccggccctggcggttggttggttgtgatccctccacatcctgtcccgtgagtcccgtcgctgacgagagagaacgaggaggagccatgggggacacctaccgcgaccccgtcgaccacctgcatacgacgcggccgctggccggcgagtcactgatcgacgtgctgcactggcctgggtacctgttggtggtggcgggggtgatcggtggtgtcggatctcttgctgccttcggcaccggccatcacgtcgaaggcatggtcgccggcgtcgcggcgctcgtcgtcacggtggccgggctggtgtggctggccgtcgagcaccggcgggtacgcaggatcgccgagcggtggtacgccgaacaccccgaggtaccacgccaacggctggccagctagcagtgccggctggcatctcaccgcaaaaccgggcgacggttttgttttaccggtggcgtcgacggggtatcaggtgtgaacaatgacgagtactggccttgccgcgtcggcgctgtcaccccatcatcggggacaggatcacgaaggcaccgacatagattgctgcagcgaccgcgatcaaaaccaccaaggtgatcccggcgatcaccgcgatgcgccggagccggcgtgcccggattgtgtcggtcacgtccgcctcgtccatggctggttgaatacccggtggcgaccatgaccaaccggttagaacgcgcggcccaaaacgggcctccgggaggcgatcggaaagggaccgaaatcgacagccaaatcgggacccaaatcagtagtagtagtgtcggtcaaaaattgccgggaggccacatgagcgatgccgatgcgcgtcccaacaggcaccaacgcggcgaccgcgccgtcgagctgaaggttgctgcgcgcttggagaatctggcgatcctgcgtaccctggtcggcgccatcggcaccttcgaggacttggatttcgatgcggtcgccgacctgagactggcggtcgacgaagtgtgtacccggctgatccgttccgccacaccgaacgcgaccttgacgctggtggtcgacccgcgtgacgacgaactcgtggtggaggcgtccgcgatgtgcgacacccacgacgtcgtggcgccgggcagcttcagctggcatgtgctgacgtcgctggccgacgacgtccagactttccacgacggccgcatgcccgacgccgccggcagtgtgttcggcattgtgttgacggcccgacgggcggcctctggcaggtgacgccgcgtgctgccggcggttctgcttcacggccgaacgaatacgccgatgtcccggagatgtttcgtgagttggccggttttgaccccgcctcaccggatttccagcgccaccgcgacaagatcgtggagcgctgcctgccgctggccgatcacatcgcccggcggttcgagggacgcggcgaaccccgcgacgacctgattcaggtcgcccgggtcggactggtcaacgcggtagtccgcttcgacgtcgagaccgggtcggatttcgtttcgttcgccgtgcccaccatcatgggggaagtccggcggcacttccgggacaacagttggtcagtcaaggttcctcgccggctgaaggaactgcacctgcggttgggcaccgccaccgccgagttgtcgcagcggctcggcagggcgcccaccgccactgaactcgccgccgaactcgggatggaccgcggcgaggtggtcgaggggctggtggcgggcagctcttacaacacgctgtccatcgacagcggtggtggtaacgaagacgacgacgcccgtgccatcgcggacaccctcggcgacatggatgccggcctggaccggatcgaagatcgcgaggcgctgcgcccgctgctcgaggcgctacccgagcgcgagcgaacggtgttgatcctcaggtttttcgagtcgatgacgcagacccagatcgccgagcgggtcggcatctcccagatgcacgtgtcccggctgctggccaagtcgctagcgcggctccgcgaccagctcgagtaggcgcaggtcgccgtcgggggcgccgtttaccgggttcaccggctccatgaccggcagcgcgccgtcgggatcgcaaatctccagtaaccgcgacacggcccggctcggcaccatcgcccactgggtgtccgccgccgagcagaccacgttgattcggtgaagggcggaaaacccggcagtgccaatgaattccagacgccgtaggtccaggatcagccaccggcaagacctcacgcactgctggacgtatccggccagctgatcggcattggcggcgtcgagctcaccttctacggtgatcacgccggccgacggcccatagctggcagtgaagtcagcggttccgcatttctgccaggattggatcacagacaatcgtggactccatccatcgaacattcgttggtgtcgaccacgtcgagtgtgcgctgcgtcgctttacgcagggagtttgcctccctcgcgaccctgacgcactgacaggacgtagctccgggcggctgtgaactcaacctgtttcgaggctaccgggcgggtgccggggcgacaacgttctccgatccgactcagataaacgctggtcaggccgggtttcgcgcggtaagcggctacttgatctcggcgagcaccgtgccctgggtgatggctgccccggcttcgaccgccagtccggtgatgacgccgtctttgtgcgcggtgaccgggttctccatcttcatcgcctccaggaccaccaccagatcgcccgtcaccacttcctgaccttcttcgaccgcgaccttcaccacggtgccctgcatgggtgcggtcacggcgtcgccggaggctgccgcaccgctgtgggcgccacgtttgcgcggcttgggcttgcgccggatgacgccgaccgggtcgcagccgccgccggacagtgcgaggtcggccggcagtgacacctcgacccggcggccgtcgacctcgacgaccaccttctgccgcggccgggcgtcctcttcgtcgctcggctcgccgccggtgaagggttcgacggtgttgttccactcggtctcgatccagcgggtgtgcaccgagaagccgtgctcgtcgccgatgaacgccgggtcggacaccaccgcccggtggaaggggatgaccgtggccagaccctcgacttcgaattcggccagcgcgcggcgggcgcgggccagcgcctcggcgcggtcggcgccgtgcacgatcagcttggccagcatcgagtcgaactggccgccgatcaccgagccggtctcgacgccggagtccatacggacgcccgggcccgcgggcgggtggaacttggtcaccgggccgggggcgggcaggaagccccgcccggcggcctcgccgttgatccggaactcgatggcgtgcccgcgcggggtggggtcctcggtgatgtcgagcgtctcgccgttggcgatcttgaactgctgcaacaccaggtcgatgccggcggtt

SEQ ID NO: 21 - DNA, 5048 bp, Mycobacterium kansasii type V
ggcgatggcgcgcttcgtcgagaccttcgtcagggtgttgggagacccggcgctaccgcatctgttcttcgtcgaaggcggcgctttggcggtggagaacgccctcaaggtcgcattcgactggaaaagccgccacaaccaggcgcgcggcatcgatccggcgctgggcacccgggtgctgcacttgagcggggcatttcacggccgcagcggctacaccctgtcgctcaccagcaccaagccggtcaccgtggcccgcttcccgaaattcgactggccgcgcgtcgacgcaccgcatatccgaccgggtttaggcgagtcggccatggatgcgctggaggccgaggcgctgcggcaggcccgcgcggcattcgaggcgcatccccacgacatcgcctgtttcatcgccgagcccatccagggcgaaggcggcgaccgccacttccggcccgagttcttcgcggcgatgcgccggttgtgtgacgaatacgatgcgctgctgattttcgacgaggtacagaccggctgtgggatcaccggaaccccttgggcttaccagcagttgggcgtggcgcccgatgtcgtggccttcggcaagaagacgcaggtgtgcggggtgatggcaggccgccgcgtcgacgaggtcgccgacaacgtgtttgccgtcaagtcgcggctcaactcgacgtggggcggaaacctggtcgacatggtgcgggcccggcgcatcctggaggtgatcgaaaacgacgggctcttcgaacatgcggcccggcagggccaccacctgcgcgcccggctcgacgagcttgcccaggagttcccgggcctggttctggatccgcgcggccgggggctgatgtgtgccttcagcctgccgaccaccgcggaccgtgacgacgtgatccgccggttgtggcaacgcgcggtgatcgtgctgccggccggtgacgacggggtgcgcttccgtccggcgttgaccgtcacgcgcgccgagatcgatgccgcgatcgccggtgtacgtgccgcattgacggctgtgagacggctgtgacctagtcggacctagtcggacctagtcgcaccgtttacctgggctgaccgcggggtatggaaacgttgtactccgcgaacgcgggatttggggttcaggatgcagaaggcacgcgaacgatcacccggtgaccgattgggacaggacgacgccgaggttcgcgccgccgtccggttcgcagtcctggccgccggcgctggtgtggggtttgtcatcatggcggccttgtgggtcagcacgtgcggcggcgcggccgtggacacggtggcctgtggcccaccggagcggaccctgctggccttcggcggcccgctgatcctgttggccggtggaatctgggccttcatccgcacctatcaggtgtggcgcgcccgcggtacctggtggggatggcacggcgccggatggttcttgttgacgctgatggtggtggctgtgtccatgggcgtgcctcccatcgccggcccggcactggcggttagttggctctgaccccgccatcctgtcccgcgagtccggccgctgacgagtgagaacgaggaggagccatgggggacacctaccgcgaccccgtcgaccacctgcatacgacgcggccgctggccggcgagtcactgatcgacgtgctgcactggccccgggtatctgctggtggtggccggggttatcggcggtgtcggatctcttgccgccttcggcaccgggcataactcccagggcatggtcgccggtgtcgcggcgctcgtggtcacggtggccgggctggtgtggctggccgccgagcaccggcgggtgcgccgaatcgccgagcggtggtatgcggaacaccccgaggtaccgcgccaacggctggccagctagcagcttccggtgccggctggcgcctcactgcaaaaaaccgggcgacggttttgttttacgggtggcgccgacggggtatcagttgtgaaccatgacgagtacgggctttgccgcgtcggcgccgtcaccccatcatcggggacagaatcacgaaggccccgacatagatcgctgcagcgatcgcgatcaacaccaccaaggtgatcccggcgatcaccgcgatgcgccggagccggcgcgtccggattgtgtcggtcacgtccgcctcgtccatggctggttgaatacccggtggcggccatgaccaaccggttagagcgcgcggcccaaaacgggcctccgggaggcgatcggaaagggaccgaaatcgacagccaaatcgggacccaaatcagtagtagtagtgtcggtcaaaaattgccgggaggccacatgagcgatgccgacgcgcgtcccaacaggcaccaacgcggcgaccgcgccgtcgagctgaacgttgctgcgcgcttggagaatctggcgatcctgcgtaccctggtcggcgccatcggcaccttcgaagacttggatttcgacgcggtcgccgacctgagactggccgtcgacgaagtgtgtacccggcttatccgttccgccacaccgaacgcgaccttgacgctggtggtcgacccgcgcgacgacgaactcgtggtggaggcgtccgcgatgtgcgacacccacgacgtcgtggcaccgggcagcttcagctggcatgtcctgacgtcgctggccgacgacgtccagactttccacgacggtcgcatgcccgacgccgccggcagtgtgttcggcattgtgttgacggcccgacgggcggccgctggcaggtgacgccgcgtgctgccggcggttctgcttcacggcccaacgaatacgccgatgtcccggagatgtttcgtgagttggccggttttgaccccgactcaccggatttccagcgccaccgcgacaacatcgtggagcgctgcctgccgctggccgatcacatcgcccggcggttcgagggacgcggcgaaccccgcgacgacctgattcaggtcgcccgggtcggactggtcaacgcggtagtccgcttcgacgtcgagaccgggtcggacttcgtctcgttcgccgtgcccaccatcatgggggaagtccggcggcacttccgggacaacagttggtcagtcaaggttcctcgccggctgaaggaactacacctgcggttgggcaccgccaccgccgagttgtcgcagcggctcggcagggcacccaccgcaaccgaacttgccgccgaactcggtatggaccgcggcgaggtcgtcgaagggctggtggcgggcagctcttacaacacactgtccatcgacagcggtggtggtaacgaagacgacgacgcccgtgccatcgcggacaccctcggcgacatcgacgccggcctggaccggatcgaagatcgcgagtcgctacgcccgttgctcgaggcgctgcccgagcgcgagcgaacggtcttgatcctcaggtttttcgagtcgatgacgcagacccagatcgccgagcgggtcggcatctcccagatgcacgtgtcccggctgctcgccaagtcgctagcgcggctccgcgaccagctcgagtaggcgcagatcgccgtcgggggcaccgttcaccgggttcaccggctccatgaccggcagcgcgccgtcgggatcgcaaatctccagtaaccgcgacacggcccggctcggcaccatcgcccactgggtgtccgccgccgagcagaccacgttgattcggtgaagagcggaaaacccggcagtcccaataaattccaggcgccgtaggtccagggtcagccaccggcaatacctcacgcactgctggacgtatccggcgagctgatcggcgttggcggcgtcgagctcaccttctacggtgaccacgccggccgacggaccatagctggcagtgaagtcagcggttccgcatttctgccaggattggatcacagacaatcgtggactccatccatcgaacattcgttggtgtcgaccacgtcgagtgtgcgctgtgcggcttacgcagggagtttgcctccctcgcgaccctgacgcactgacaggacgtggctccgggcggctgtgaactcaacctgttttgaggctacccggcgggtgccggggcgacaacgttctccgatccgactcagagaatcgctggtcaggcaggggttggcgcggtgagcggctacttgatctcggccagcaccgttccctgggtgatggcggccccggcttcgaccgccagcccggtgatgacgccgtccttatgcgcggtgaccgggttctccatcttcatcgcctccaggacgaccacgaggtcgcccgtcgccacttcctgcccttcttcgaccgcgaccttcaccacggtgccctgcatgggcgcggtaacggcgtcgccggaggctgccgcaccgctgtgggcgccacgcttgcgcggcttgggcttgcgccggataacaccgaccgggtcgcacccgccgccgccggacagtgcgaggtcggccggcagtgacacctcgacccggcggccgtcgacctcgacgaccaccttctgccgcggccgggcgtcctcttcgtcgctcggctcgctgccggtgaagggttcgacggtgttgttccactcggtctcgatccagcgggtgtgcaccgagaagccgtgctcgtcgccgatgaatgccgggtcggacaccaccgcccggtggaaggggatcaccgtcgccagaccctcgacttcgaattcggccagcgcgcggcgggcgcgggccagcgcctcggcacggtcggcgccgtgaacgatcagcttggccagcatcgagtcgaactggccgccaatcaccgagccggtctcgacgccggagtccatacggacgcccgggcccgcgggcgggtggaacttggtcaccgggccgggcgcgggcaggaagccccgcccggcgtcctcgccgttgatccggaactcgatggcgtgcccgcgcggggtggggtcctcggtgatgtcgagcttgtcgccgttggcgatcttgaactgctgcagtaccaagtcgatgccggcggtt

SEQ ID NO: 22 - DNA, 20 bp, Artificial
  Primer
acgagtgagaacgaggagga

SEQ ID NO: 23 - DNA, 20 bp, Artificial
  Primer
atgttcggcataccaccgtt

SEQ ID NO: 24 - DNA, 20 bp, Artificial
  Primer
tgagaacgaggaggagccat

SEQ ID NO: 25 - DNA, 20 bp, Artificial
  Primer
tgttcggcataccaccgttc

SEQ ID NO: 26 - DNA, 21 bp, Artificial
  Primer
ctgacgagtgagaacgaggag

SEQ ID NO: 27 - DNA, 19 bp, Artificial
  Primer
gatccgacaccgccgataa

SEQ ID NO: 28 - DNA, 20 bp, Artificial
  Primer
ttatcggcggtgtcggatct

SEQ ID NO: 29 - DNA, 19 bp, Artificial
  Primer
ttcggcataccaccgttcg

SEQ ID NO: 30 - DNA, 19 bp, Artificial
  Primer
tcgctgacgagtgagaacg

SEQ ID NO: 31 - DNA, 20 bp, Artificial
  Primer
gagatccgacaccgccgata

SEQ ID NO: 32 - DNA, 20 bp, Artificial
  Primer
tcgctgacgagtgagaacga

SEQ ID NO: 33 - DNA, 19 bp, Artificial
  Primer
gtatgcaggtggtcgacgg

SEQ ID NO: 34 - DNA, 20 bp, Artificial
  Primer
tatcggcggtgtcggatctc

SEQ ID NO: 35 - DNA, 20 bp, Artificial
  Primer
gttcggcataccaccgttcg

SEQ ID NO: 36 - DNA, 19 bp, Artificial
  Primer
atgactcccagggcatggt

SEQ ID NO: 37 - DNA, 21 bp, Artificial
  Primer
gatgttcggcataccaccgtt

SEQ ID NO: 38 - DNA, 27 bp, Artificial
  Probe
accggatgtctgccgccgagcagacca

SEQ ID NO: 39 - DNA, 31 bp, Artificial
  Probe
ttggcggcgtcgagctcaccttccacggtga

SEQ ID NO: 40 - DNA, 30 bp, Artificial
  Probe
cagggagtttgccttcctggcgaccctgac

SEQ ID NO: 41 - DNA, 20 bp, Artificial
  Tag
gacaacggagacagagccaa

SEQ ID NO: 42 - DNA, 20 bp, Artificial
  Tag
atgctaccgtatgcccagtg

SEQ ID NO: 43 - DNA, 20 bp, Artificial
  Tag
ttggctctgtctccgttgtc

SEQ ID NO: 44 - DNA, 20 bp, Artificial
  Tag
cactgggcatacggtagcat